European Patent Application EP 4 155 410 A9, published July 19, 2023. Title: NUCLEIC ACID CONSTRUCT, RECOMBINANT INFLUENZA VIRUS, METHOD FOR PREPARING RECOMBINANT INFLUENZA VIRUS, COMPOSITION, AND USE. Applicant: FUNDACAO OSWALDO CRUZ. The sequence listing filed with the application follows.

SEQUENCE LISTING (9 sequences)

SEQ ID NO: 1 - DNA, 3142 bp, Artificial sequence
  Plasmid pPRNA166x178
agcaaaagcaggagtttaactaaatccaaaccagaaaataataaccattggatcgatctgtctagtagtcggaataattagcctaatattgcaaataggaaatataatctcaatctagattagccattcaattcaaaccggaaatcaaaaccatactggaatctactctagactcgagagctagcgtcgactgcttctgggttgaattaatcagggggctacctgaggaggacgcaatctggactagtgggagcatcatttctttttgtggtgtgaatggtgatactgtagattggtcttggccagacggtgctgagttgccgttcaccattgacaagtagtttgttcaaaaaactccttgtttctactaataacccggcggcccaaaatgccgactcggagcgaaagatatacctcccccggggccgggaggtcgcgtcaccgaccacgccgccggcccaggcgacgcgcgacacggacacctgtccccaaaaacgccaccatcgcagccacacacggagcgcccggggccctctggtcaaccccaggacacacgcgggagcagcgccgggccggggacgccctcccggccgcccgtgccacacgcaggggccggcccgtaagcttggcgtaatcatggtcatagctgtttcctgtgtgaaattgttatccgctcacaattccacacaacatacgagccggaagcataaagtgtaaagcctggggtgcctaatgagtgagctaactcacattaattgcgttgcgctcactgcccgctttccagtcgggaaacctgtcgtgccagctgcattaatgaatcggccaacgcgcggggagaggcggtttgcgtattgggcgctcttccgcttcctcgctcactgactcgctgcgctcggtcgttcggctgcggcgagcggtatcagctcactcaaaggcggtaatacggttatccacagaatcaggggataacgcaggaaagaacatgtgagcaaaaggccagcaaaaggccaggaaccgtaaaaaggccgcgttgctggcgtttttccataggctccgcccccctgacgagcatcacaaaaatcgacgctcaagtcagaggtggcgaaacccgacaggactataaagataccaggcgtttccccctggaagctccctcgtgcgctctcctgttccgaccctgccgcttaccggatacctgtccgcctttctcccttcgggaagcgtggcgctttctcatagctcacgctgtaggtatctcagttcggtgtaggtcgttcgctccaagctgggctgtgtgcacgaaccccccgttcagcccgaccgctgcgccttatccggtaactatcgtcttgagtccaacccggtaagacacgacttatcgccactggcagcagccactggtaacaggattagcagagcgaggtatgtaggcggtgctacagagttcttgaagtggtggcctaactacggctacactagaaggacagtatttggtatctgcgctctgctgaagccagttaccttcggaaaaagagttggtagctcttgatccggcaaacaaaccaccgctggtagcggtggtttttttgtttgcaagcagcagattacgcgcagaaaaaaaggatctcaagaagatcctttgatcttttctacggggtctgacgctcagtggaacgaaaactcacgttaagggattttggtcatgagattatcaaaaaggatcttcacctagatccttttaaattaaaaatgaagttttaaatcaatctaaagtatatatgagtaaacttggtctgacagttaccaatgcttaatcagtgaggcacctatctcagcgatctgtctatttcgttcatccatagttgcctgactccccgtcgtgtagataactacgatacgggagggcttaccatctggccccagtgctgcaatgataccgcgagacccacgctcaccggctccagatttatcagcaataaaccagccagccggaagggccgagcgcagaagtggtcctgcaactttatccgcctccatccagtctattaattgttgccgggaagctagagtaagtagttcgccagttaatagtttgcgcaacgttgttgccattgctacaggcatcgtggtgtcacgctcgtcgtttggtatggcttcattcagctccggttcccaacgatcaaggcgagttacatgatcccccatgttgtgcaaaaaagcggttagctccttcggtcctccgatcgttgtcagaagtaagttggccgcagtgttatcactcatggttatggcagcactgcataattctcttactgtcatgccatccgtaagatgcttttctgtgactggtgagtactcaaccaagtcattctgagaatagtgtatgcggcgaccgagttgctcttgcccggcgtcaatacgggataataccgcgccacatagcagaactttaaaagtgctcatcattggaaaacgttcttcggggcgaaaactctcaaggatcttaccgctgttgagatccagttcgatgtaacccactcgtgcacccaactgatcttcagcatcttttactttcaccagcgtttctgggtgagcaaaaacaggaaggcaaaatgccgcaaaaaagggaataagggcgacacggaaatgttgaatactcatactcttcctttttcaatattattgaagcatttatcagggttattgtctcatgagcggatacatatttgaatgtatttagaaaaataaacaaataggggttccgcgcacatttccccgaaaagtgccacctgacgtctaagaaaccattattatcatgacattaacctataaaaataggcgtatcacgaggccctttcgtctcgcgcgtttcggtgatgacggtgaaaacctctgacacatgcagctcccggagacggtcacagcttgtctgtaagcggatgccgggagcagacaagcccgtcagggcgcgtcagcgggtgttggcgggtgtcggggctggcttaactatgcggcatcagagcagattgtactgagagtgcaccatatgcggtgtgaaataccgcacagatgcgtaaggagaaaataccgcatcaggcgccattcgccattcaggctgcgcaactgttgggaagggcgatcg

SEQ ID NO: 2 - DNA, 534 bp, Homo sapiens
atgttccatgtttcttttaggtatatctttggacttcctcccctgatccttgttctgttgccagtagcatcatctgattgtgatattgaaggtaaagatggcaaacaatatgagagtgttctaatggtcagcatcgatcaattattggacagcatgaaagaaattggtagcaattgcctgaataatgaatttaacttttttaaaagacatatctgtgatgctaataaggaaggtatgtttttattccgtgctgctcgcaagttgaggcaatttcttaaaatgaatagcactggtgattttgatctccacttattaaaagtttcagaaggcacaacaatactgttgaactgcactggccaggttaaaggaagaaaaccagctgccctgggtgaagcccaaccaacaaagagtttggaagaaaataaatctttaaaggaacagaaaaaactgaatgacttgtgtttcctaaagagactattacaagagataaaaacttgttggaataaaattttgatgggcactaaagaacactga

SEQ ID NO: 3 - DNA, 530 bp, Sus scrofa
atgttccatgtttcttttaggtatatcttcggaattcctcccctgatccttgttctgttgccagtagcatcatctgattgtgatattgaaggtaaagacggcggagtgtatcagaatgttctaatggtcagcatcgatgacttggacaggatgatagactttgatagcaattgcctgaataacgaacctaactttttaaaaaaacattcatgtgatgataataaggaagcttcatttttatatcgtgctgctcgaaagttgaagcaatttattaaaatgaatatcagtgaggagttcaatcaccatctatcaacagtttcacagggcacattaacactgttcaactgcaccagcaaggttaaaggaagaaaaccaccttccctgggtgaagcccaactcactaagaacttggaagaaaataaatctttaaaggaacagaaaagacagggggacttgtgtttcctaaagatactactacagaagataaaaacttgttggaataaaattttgaggggtgctaaagaatattg

SEQ ID NO: 4 - DNA, 465 bp, Mus musculus
atgttccatgtttcttttagatatatctttggaattcctccactgatccttgttctgctgcctgtcacatcatctgagtgccacattaaagacaaagaaggtaaagcatatgagagtgtactgatgatcagcatcgatgaattggacaaaatgacaggaactgatagtaattgcccgaataatgaaccaaacttttttagaaaacatgtatgtgatgatacaaaggaagctgcttttctaaatcgtgctgctcgcaagttgaagcaatttcttaaaatgaatatcagtgaagaattcaatgtccacttactaacagtatcacaaggcacacaaacactggtgaactgcacaagtaaggaagaaaaaaacgtaaaggaacagaaaaagaatgatgcatgtttcctaaagagactactgagagaaataaaaacttgttggaataaaattttgaagggcagtatataa

SEQ ID NO: 5 - protein, 177 aa, Homo sapiens
MFHVSFRYIFGLPPLILVLLPVASSDCDIEGKDGKQYESVLMVSIDQLLDSMKEIGSNCLNNEFNFFKRHICDANKEGMFLFRAARKLRQFLKMNSTGDFDLHLLKVSEGTTILLNCTGQVKGRKPAALGEAQPTKSLEENKSLKEQKKLNDLCFLKRLLQEIKTCWNKILMGTKEH

SEQ ID NO: 6 - protein, 154 aa, Mus musculus
MFHVSFRYIFGIPPLILVLLPVTSSECHIKDKEGKAYESVLMISIDELDKMTGTDSNCPNNEPNFFRKHVCDDTKEAAFLNRAARKLKQFLKMNISEEFNVHLLTVSQGTQTLVNCTSKEEKNVKEQKKNDACFLKRLLREIKTCWNKILKGSI

SEQ ID NO: 7 - protein, 176 aa, Sus scrofa
MFHVSFRYIFGIPPLILVLLPVASSDCDIEGKDGGVYQNVLMVSIDDLDRMIDFDSNCLNNEPNFLKKHSCDDNKEASFLYRAARKLKQFIKMNISEEFNHHLSTVSQGTLTLFNCTSKVKGRKPPSLGEAQLTKNLEENKSLKEQKRQGDLCFLKILLQKIKTCWNKILRGAKEY

SEQ ID NO: 8 - DNA, 465 bp, Mus musculus
atgttccacgtgtcttttagatacatttttgggattccacctctgattctggtcctgctgcctgtcacctcctctgagtgtcatattaaggacaaagagggcaaagcttacgaaagcgtgctgatgatctccattgacgagctggataagatgaccggaacagattctaactgccccaacaatgagcctaatttctttcggaaacacgtctgtgacgataccaaggaagccgctttcctgaacagggcagccagaaagctgaaacagttcctgaagatgaacatctctgaggagttcaacgtgcatctgctgacagtcagtcagggcactcagaccctggtgaattgcactagcaaggaggagaagaacgtgaaggaacagaagaaaaatgacgcctgttttctgaagaggctgctgcgggaaatcaagacctgctggaacaaaatcctgaaaggctcaatctga

SEQ ID NO: 9 - DNA, 3825 bp, Artificial sequence
  Plasmid pPRNA166-IL7-178
agcaaaagcaggagtttaactaaatccaaaccagaaaataataaccattggatcgatctgtctagtagtcggaataattagcctaatattgcaaataggaaatataatctcaatctagattagccattcaattcaaaccggaaatcaaaaccatactggaatctactctagactcgagcgcgccaccatgttccacgtgtcttttagatacatttttgggattccacctctgattctggtcctgctgcctgtcacctcctctgagtgtcatattaaggacaaagagggcaaagcttacgaaagcgtgctgatgatctccattgacgagctggataagatgaccggaacagattctaactgccccaacaatgagcctaatttctttcggaaacacgtctgtgacgataccaaggaagccgctttcctgaacagggcagccagaaagctgaaacagttcctgaagatgaacatctctgaggagttcaacgtgcatctgctgacagtcagtcagggcactcagaccctggtgaattgcactagcaaggaggagaagaacgtgaaggaacagaagaaaaatgacgcctgttttctgaagaggctgctgcgggaaatcaagacctgctggaacaaaatcctgaaaggctcaatctgagctagcgtcgactgcttctgggttgaattaatcagggggctacctgaggaggacgcaatctggactagtgggagcatcatttctttttgtggtgtgaatggtgatactgtagattggtcttggccagacggtgctgagttgccgttcaccattgacaagtagtttgttcaaaaaactccttgtttctactaataacccggcggcccaaaatgccgactcggagcgaaagatatacctcccccggggccgggaggtcgcgtcaccgaccacgccgccggcccaggcgacgcgcgacacggacacctgtccccaaaaacgccaccatcgcagccacacacggagcgcccggggccctctggtcaaccccaggacacacgcgggagcagcgccgggccggggacgccctcccggccgcccgtgccacacgcaggggccggcccgtaagcttggcgtaatcatggtcatagctgtttcctgtgtgaaattgttatccgctcacaattccacacaacatacgagccggaagcataaagtgtaaagcctggggtgcctaatgagtgagctaactcacattaattgcgttgcgctcactgcccgctttccagtcgggaaacctgtcgtgccagctgcattaatgaatcggccaacgcgcggggagaggcggtttgcgtattgggcgctcttccgcttcctcgctcactgactcgctgcgctcggtcgttcggctgcggcgagcggtatcagctcactcaaaggcggtaatacggttatccacagaatcaggggataacgcaggaaagaacatgtgagcaaaaggccagcaaaaggccaggaaccgtaaaaaggccgcgttgctggcgtttttccataggctccgcccccctgacgagcatcacaaaaatcgacgctcaagtcagaggtggcgaaacccgacaggactataaagataccaggcgtttccccctggaagctccctcgtgcgctctcctgttccgaccctgccgcttaccggatacctgtccgcctttctcccttcgggaagcgtggcgctttctcatagctcacgctgtaggtatctcagttcggtgtaggtcgttcgctccaagctgggctgtgtgcacgaaccccccgttcagcccgaccgctgcgccttatccggtaactatcgtcttgagtccaacccggtaagacacgacttatcgccactggcagcagccactggtaacaggattagcagagcgaggtatgtaggcggtgctacagagttcttgaagtggtggcctaactacggctacactagaaggacagtatttggtatctgcgctctgctgaagccagttaccttcggaaaaagagttggtagctcttgatccggcaaacaaaccaccgctggtagcggtggtttttttgtttgcaagcagcagattacgcgcagaaaaaaaggatctcaagaagatcctttgatcttttctacggggtctgacgctcagtggaacgaaaactcacgttaagggattttggtcatgagattatcaaaaaggatcttcacctagatccttttaaattaaaaatgaagttttaaatcaatctaaagtatatatgagtaaacttggtctgacagttaccaatgcttaatcagtgaggcacctatctcagcgatctgtctatttcgttcatccatagttgcctgactccccgtcgtgtagataactacgatacgggagggcttaccatctggccccagtgctgcaatgataccgcgagacccacgctcaccggctccagatttatcagcaataaaccagccagccggaagggccgagcgcagaagtggtcctgcaactttatccgcctccatccagtctattaattgttgccgggaagctagagtaagtagttcgccagttaatagtttgcgcaacgttgttgccattgctacaggcatcgtggtgtcacgctcgtcgtttggtatggcttcattcagctccggttcccaacgatcaaggcgagttacatgatcccccatgttgtgcaaaaaagcggttagctccttcggtcctccgatcgttgtcagaagtaagttggccgcagtgttatcactcatggttatggcagcactgcataattctcttactgtcatgccatccgtaagatgcttttctgtgactggtgagtactcaaccaagtcattctgagaatagtgtatgcggcgaccgagttgctcttgcccggcgtcaatacgggataataccgcgccacatagcagaactttaaaagtgctcatcattggaaaacgttcttcggggcgaaaactctcaaggatcttaccgctgttgagatccagttcgatgtaacccactcgtgcacccaactgatcttcagcatcttttactttcaccagcgtttctgggtgagcaaaaacaggaaggcaaaatgccgcaaaaaagggaataagggcgacacggaaatgttgaatactcatactcttcctttttcaatattattgaagcatttatcagggttattgtctcatgagcggatacatatttgaatgtatttagaaaaataaacaaataggggttccgcgcacatttccccgaaaagtgccacctgacgtctaagaaaccattattatcatgacattaacctataaaaataggcgtatcacgaggccctttcgtctcgcgcgtttcggtgatgacggtgaaaacctctgacacatgcagctcccggagacggtcacagcttgtctgtaagcggatgccgggagcagacaagcccgtcagggcgcgtcagcgggtgttggcgggtgtcggggctggcttaactatgcggcatcagagcagattgtactgagagtgcaccatatgcggtgtgaaataccgcacagatgcgtaaggagaaaataccgcatcaggcgccattcgccattcaggctgcgcaactgttgggaagggcgatcggtgcgggcctcttcgctattacgccagctggcgaaagggggatgtgctgcaaggcgattaagttgggtaacgccagggttttcccagtcacgacgttgtaaaacgacggccagtgaattcgagctcgtcccattcgccattaccgaggggacggtcccctcggaatgttgcccagccggcgccagcgaggaggctgggaccatgccggcc